European Patent Specification EP 3 426 684 B1, published October 9, 2024. Title: MULTIPLEXED IMMUNOHISTOCHEMISTRY USING RECOMBINANT ANTIBODIES WITH EPITOPE TAGS. Applicant: VENTANA MEDICAL SYSTEMS TANG, Lei MCEHHINNY, Abgail ZHANG, Wenjun FARRELL, Mike HUBBARD, Antony COUTO, Joseph BHAUMIK, Srabani URIBE, Diana HAO, Junshan JONES, Tobin ZHU, Yifei DAY, Bill. The sequence listing filed with the application follows.

SEQUENCE LISTING (32 sequences)

SEQ ID NO: 1 - protein, 11 aa, Artificial Sequence
  Synthetic:  VSV Epitope tag
YTDIEMNRLGK

SEQ ID NO: 2 - protein, 6 aa, Artificial Sequence
  Synthetic:  AU5 Epitope tag
TDFYLK

SEQ ID NO: 3 - protein, 13 aa, Artificial Sequence
  Synthetic:  E Epitope tag
GAPVPYPDPLEPR

SEQ ID NO: 4 - protein, 14 aa, Artificial Sequence
  Synthetic:  V5 Epitope tag
GKPIPNPLLGLDST

SEQ ID NO: 5 - protein, 9 aa, Artificial Sequence
  Synthetic:  HA Epitope tag
YPYDVPDYA

SEQ ID NO: 6 - protein, 12 aa, Artificial Sequence
  Synthetic:  E2 Epitope tag
GVSSTSSDFRDR

SEQ ID NO: 7 - protein, 11 aa, Artificial Sequence
  Synthetic:  KT3 Epitope tag
KPPTPPPEPET

SEQ ID NO: 8 - protein, 6 aa, Artificial Sequence
  Synthetic:  AU1 Epitope tag
DTYRYI

SEQ ID NO: 9 - protein, 14 aa, Artificial Sequence
  Synthetic:  OLLAS Epitope tag
SGFANELGPRLMGK

SEQ ID NO: 10 - protein, 31 aa, Artificial Sequence
  Synthetic:  Repeated portion of AA sequence of spacer
GRSSGQPKAPSVPNSASHSGSAPNTSSAPGS

SEQ ID NO: 11 - protein, 31 aa, Artificial Sequence
  Synthetic:  Repeated portion of AA sequence of spacer
SASSGQPKAPSVPNSASHSGSAPNTSSAPGS

SEQ ID NO: 12 - protein, 31 aa, Artificial Sequence
  Synthetic:  Repeated portion of AA sequence of spacer
SRSVGQPKAPSVPNSASHSGSAPNTSSAPGS

SEQ ID NO: 13 - protein, 31 aa, Artificial Sequence
  Synthetic:  Repeated portion of AA sequence of spacer
DISSGQPKAPSVPNSASHSGSAPNTSSAPGS

SEQ ID NO: 14 - protein, 31 aa, Artificial Sequence
  Synthetic:  Repeated portion of AA sequence of spacer
GASSGQPKAPSVPNSASHSGSAPNTSSAPGS

SEQ ID NO: 15 - DNA, 631 bp, Artificial Sequence
  Synthetic:  4 VSV nucleic acid sequence
agcggccgcagcagtggacaaccaaaagcaccatcagtaccgaactccgcctcgcactctggcagcgcgcctaatacaagttcagctccggggtcctatactgatattgaaatgaatcggcttggcaaaagcgcttctagcggccagcctaaagctccgagtgtccccaattcagcgtcccattcggggtctgccccaaacacgtcgtccgcacccggttcatacaccgacatcgagatgaaccgcctcgggaagtcgcgaagcgttggacaaccgaaagcaccctcggtgccaaactccgcatcacatagtggcagcgcccccaatacaagttcagcgccagggtcctatacagatattgaaatgaatagactgggaaaagatatctctagcgggcagcctaaggctccctcagttcccaactctgcttcccactcggggtctgcgccaaatacctctagcgcccctggctcttacacagacattgagatgaatcggcttggcaagggcgccagtagcggccaacctaaagcaccttcagtgccaaattccgcatcgcattctgggtcggcccccaatacttcctcagcgccagggagcagcagtggcgcctagtagggccggcaaggcc

SEQ ID NO: 16 - protein, 209 aa, Artificial Sequence
  Synthetic:  4 VSV amino acid sequence
  misc_feature (204)..(205): Location of stop codon
SGRSSGQPKAPSVPNSASHSGSAPNTSSAPGSYTDIEMNRLGKSASSGQPKAPSVPNSASHSGSAPNTSSAPGSYTDIEMNRLGKSRSVGQPKAPSVPNSASHSGSAPNTSSAPGSYTDIEMNRLGKDISSGQPKAPSVPNSASHSGSAPNTSSAPGSYTDIEMNRLGKGASSGQPKAPSVPNSASHSGSAPNTSSAPGSSSGAGRQGR

SEQ ID NO: 17 - DNA, 571 bp, Artificial Sequence
  Synthetic:  4 AU5 nucleic acid sequence
agcggccgcagcagtggacaaccaaaagcaccatcagtaccgaactccgcctcgcactctggcagcgcgcctaatacaagttcagctccggggtccactgatttttatttgaaaagcgcttctagcggccagcctaaagctccgagtgtccccaattcagcgtcccattcggggtctgccccaaacacgtcgtccgcacccggttcaaccgacttctacctcaagtcgcgaagcgttggacaaccgaaagcaccctcggtgccaaactccgcatcacatagtggcagcgcccccaatacaagttcagcgccagggtccacagatttttatctgaaagatatctctagcgggcagcctaaggctccctcagttcccaactctgcttcccactcggggtctgcgccaaatacctctagcgcccctggctctacagatttttacttgaagggcgccagtagcggccaacctaaagcaccttcagtgccaaattccgcatcgcattctgggtcggcccccaatacttcctcagcgccagggagcagcagtggcgcctagtagggccggcaaggcc

SEQ ID NO: 18 - protein, 188 aa, Artificial Sequence
  Synthetic:  4 AU5 amino acid sequence
  misc_feature (184)..(185): Location of stop codon
SGRSSGQPKAPSVPNSASHSGSAPNTSSAPGSTDFYLKSASSGQPKAPSVPNSASHSGSAPNTSSAPGSTDFYLKSRSVGQPKAPSVPNSASHSGSAPNTSSAPGSTDFYLKDISSGQPKAPSVPNSASHSGSAPNTSSAPGSTDFYLKGASSGQPKAPSVPNSASHSGSAPNTSSAPGSSSGAGRQG

SEQ ID NO: 19 - DNA, 655 bp, Artificial Sequence
  Synthetic:  4 E nucleic acid sequence
agcggccgcagcagtggacaaccaaaagcaccatcagtaccgaactccgcctcgcactctggcagcgcgcctaatacaagttcagctccggggtccggcgctcctgttccttatcccgatccattggaacctcgcagcgcttctagcggccagcctaaagctccgagtgtccccaattcagcgtcccattcggggtctgccccaaacacgtcgtccgcacccggttcaggggcaccagtgccctaccctgatccactcgaaccccggtcgcgaagcgttggacaaccgaaagcaccctcggtgccaaactccgcatcacatagtggcagcgcccccaatacaagttcagcgccagggtccggggcccccgtcccttatccagatcccctggaacctagggatatctctagcgggcagcctaaggctccctcagttcccaactctgcttcccactcggggtctgcgccaaatacctctagcgcccctggctctggagctccagttccctatcctgacccactggagcctagaggcgccagtagcggccaacctaaagcaccttcagtgccaaattccgcatcgcattctgggtcggcccccaatacttcctcagcgccagggagcagcagtggcgcctagtagggccggcaaggcc

SEQ ID NO: 20 - protein, 216 aa, Artificial Sequence
  Synthetic:  4 E amino acid sequence
  misc_feature (212)..(213): Location of stop codon
SGRSSGQPKAPSVPNSASHSGSAPNTSSAPGSGAPVPYPDPLEPRSASSGQPKAPSVPNSASHSGSAPNTSSAPGSGAPVPYPDPLEPRSRSVGQPKAPSVPNSASHSGSAPNTSSAPGSGAPVPYPDPLEPRDISSGQPKAPSVPNSASHSGSAPNTSSAPGSGAPVPYPDPLEPRGASSGQPKAPSVPNSASHSGSAPNTSSAPGSSSGAGRQG

SEQ ID NO: 21 - DNA, 709 bp, Artificial Sequence
  Synthetic:  5 V5 nucleic acid sequence
agcggccgcagcagtggacaaccaaaagcaccatcagtaccgaactccgcctcgcactctggcagcgcgcctaatacaagttcagctccggggtccggtaagccaatacccaacccgctcctaggactggattcgaccagcgcttctagcggccagcctaaagctccgagtgtccccaattcagcgtcccattcggggtctgccccaaacacgtcgtccgcacccggttcagggaagccgatccctaatcctcttttaggcttggatagtacttcgcgaagcgttggacaaccgaaagcaccctcggtgccaaactccgcatcacatagtggcagcgcccccaatacaagttcagcgccagggtccggtaagcctattccaaacccactccttggtctcgactcgaccgatatctctagcgggcagcctaaggctccctcagttcccaactctgcttcccactcggggtctgcgccaaatacctctagcgcccctggctctggaaaaccaattcccaacccgttgcttggattagattcaacgggcgccagtagcggccaacctaaagcaccttcagtgccaaattccgcatcgcattctgggtcggcccccaatacttcctcagcgccagggagcggaaagccgatcccaaacccactactcggcctggacagtacgagcagtggcgcctagtagggccggcaaggcc

SEQ ID NO: 22 - protein, 234 aa, Artificial Sequence
  Synthetic:  5 V5 amino acid sequence
  misc_feature (230)..(231): Location of stop codon
SGRSSGQPKAPSVPNSASHSGSAPNTSSAPGSGKPIPNPLLGLDSTSASSGQPKAPSVPNSASHSGSAPNTSSAPGSGKPIPNPLLGLDSTSRSVGQPKAPSVPNSASHSGSAPNTSSAPGSGKPIPNPLLGLDSTDISSGQPKAPSVPNSASHSGSAPNTSSAPGSGKPIPNPLLGLDSTGASSGQPKAPSVPNSASHSGSAPNTSSAPGSGKPIPNPLLGLDSTSSGAGRQG

SEQ ID NO: 23 - DNA, 607 bp, Artificial Sequence
  Synthetic:  4 HA nucleic acid sequence
agcggccgcagcagtggacaaccaaaagcaccatcagtaccgaactccgcctcgcactctggcagcgcgcctaatacaagttcagctccggggtcctatccttacgatgttcccgattacgcttctgcttctagcggccagcctaaagctccgagtgtccccaattcagcgtcccattcggggtctgccccaaacacgtcgtccgcacccggttcatacccctatgacgtcccagattatgcatcgcgaagcgttggacaaccgaaagcaccctcggtgccaaactccgcatcacatagtggcagcgcccccaatacaagttcagcgccagggtcctatccctacgacgttcctgattatgccgatatctctagcgggcagcctaaggctccctcagttcccaactctgcttcccactcggggtctgcgccaaatacctctagcgcccctggctcttatccctacgacgtgccagattacgcaggcgccagtagcggccaacctaaagcaccttcagtgccaaattccgcatcgcattctgggtcggcccccaatacttcctcagcgccagggagcagcagtggcgcctagtagggccggcaaggcc

SEQ ID NO: 24 - protein, 200 aa, Artificial Sequence
  Synthetic:  4 HA amino acid sequence
  misc_feature (196)..(197): Location of stop codon
SGRSSGQPKAPSVPNSASHSGSAPNTSSAPGSYPYDVPDYASASSGQPKAPSVPNSASHSGSAPNTSSAPGSYPYDVPDYASRSVGQPKAPSVPNSASHSGSAPNTSSAPGSYPYDVPDYADISSGQPKAPSVPNSASHSGSAPNTSSAPGSYPYDVPDYAGASSGQPKAPSVPNSASHSGSAPNTSSAPGSSSGAGRQG

SEQ ID NO: 25 - DNA, 643 bp, Artificial Sequence
  Synthetic:  4 E2 nucleic acid sequence
agcggccgcagcagtggacaaccaaaagcaccatcagtaccgaactccgcctcgcactctggcagcgcgcctaatacaagttcagctccggggtccggcgtttcttcaacttcctctgattttcgcgacagaagcgcttctagcggccagcctaaagctccgagtgtccccaattcagcgtcccattcggggtctgccccaaacacgtcgtccgcacccggttcaggagtcagcagtacctcatctgacttccgggatcggtcgcgaagcgttggacaaccgaaagcaccctcggtgccaaactccgcatcacatagtggcagcgcccccaatacaagttcagcgccagggtccggggtgagctctacaagttcagattttagagaccgcgatatctctagcgggcagcctaaggctccctcagttcccaactctgcttcccactcggggtctgcgccaaatacctctagcgcccctggctctggcgtgtcttccactagctctgactttcgggacaggggcgccagtagcggccaacctaaagcaccttcagtgccaaattccgcatcgcattctgggtcggcccccaatacttcctcagcgccagggagcagcagtggcgcctagtagggccggcaaggcc

SEQ ID NO: 26 - protein, 212 aa, Artificial Sequence
  Synthetic:  4 E2 amino acid sequence
  misc_feature (208)..(209): Location of stop codon
SGRSSGQPKAPSVPNSASHSGSAPNTSSAPGSGVSSTSSDFRDRSASSGQPKAPSVPNSASHSGSAPNTSSAPGSGVSSTSSDFRDRSRSVGQPKAPSVPNSASHSGSAPNTSSAPGSGVSSTSSDFRDRDISSGQPKAPSVPNSASHSGSAPNTSSAPGSGVSSTSSDFRDRGASSGQPKAPSVPNSASHSGSAPNTSSAPGSSSGAGRQG

SEQ ID NO: 27 - DNA, 637 bp, Artificial Sequence
  Synthetic:  4 KT3 nucleic acid sequence
agcggccgcagcagtggacaaccaaaagcaccatcagtaccgaactccgcctcgcactctggcagcgcgcctaatacaagttcagctccggggtccaaacctccaactcccccacctgaacctgagactagcgcttctagcggccagcctaaagctccgagtgtccccaattcagcgtcccattcggggtctgccccaaacacgtcgtccgcacccggttcaaagccacccaccccacctcccgagcccgaaacatcgcgaagcgttggacaaccgaaagcaccctcggtgccaaactccgcatcacatagtggcagcgcccccaatacaagttcagcgccagggtccaaaccacctacacctccacccgaaccagagaccgatatctctagcgggcagcctaaggctccctcagttcccaactctgcttcccactcggggtctgcgccaaatacctctagcgcccctggctctaagcctcccacaccaccccctgagcctgaaactggcgccagtagcggccaacctaaagcaccttcagtgccaaattccgcatcgcattctgggtcggcccccaatacttcctcagcgccagggagcagcagtggcgcctagtagggccggcaaggccggatcc

SEQ ID NO: 28 - protein, 208 aa, Artificial Sequence
  Synthetic:  4 KT3 amino acid sequence
  misc_feature (204)..(205): Location of stop codon
SGRSSGQPKAPSVPNSASHSGSAPNTSSAPGSKPPTPPPEPETSASSGQPKAPSVPNSASHSGSAPNTSSAPGSKPPTPPPEPETSRSVGQPKAPSVPNSASHSGSAPNTSSAPGSKPPTPPPEPETDISSGQPKAPSVPNSASHSGSAPNTSSAPGSKPPTPPPEPETGASSGQPKAPSVPNSASHSGSAPNTSSAPGSSSGAGRQG

SEQ ID NO: 29 - DNA, 673 bp, Artificial Sequence
  Synthetic:  4 OLLAS nucleic acid sequence
agcggccgcagcagtggacaaccaaaagcaccatcagtaccgaactccgcctcgcactctggcagcgcgcctaatacaagttcagctccggggtccagtggctttgctaatgaattgggccctagattgatgggaaagagcgcttctagcggccagcctaaagctccgagtgtccccaattcagcgtcccattcggggtctgccccaaacacgtcgtccgcacccggttcatcagggttcgcaaacgagctcgggccaagacttatgggcaaatcgcgaagcgttggacaaccgaaagcaccctcggtgccaaactccgcatcacatagtggcagcgcccccaatacaagttcagcgccagggtcctccggctttgccaatgagctgggaccccgccttatgggcaaagatatctctagcgggcagcctaaggctccctcagttcccaactctgcttcccactcggggtctgcgccaaatacctctagcgcccctggctcttctgggtttgcaaatgagttggggcctaggttgatgggcaagggcgccagtagcggccaacctaaagcaccttcagtgccaaattccgcatcgcattctgggtcggcccccaatacttcctcagcgccagggagcagcagtggcgcctagtagggccggcaaggccggatcc

SEQ ID NO: 30 - protein, 220 aa, Artificial Sequence
  Synthetic:  4 OLLAS amino acid sequence
  misc_feature (216)..(217): Location of stop codon
SGRSSGQPKAPSVPNSASHSGSAPNTSSAPGSSGFANELGPRLMGKSASSGQPKAPSVPNSASHSGSAPNTSSAPGSSGFANELGPRLMGKSRSVGQPKAPSVPNSASHSGSAPNTSSAPGSSGFANELGPRLMGKDISSGQPKAPSVPNSASHSGSAPNTSSAPGSSGFANELGPRLMGKGASSGQPKAPSVPNSASHSGSAPNTSSAPGSSSGAGRQG

SEQ ID NO: 31 - DNA, 577 bp, Artificial Sequence
  Synthetic:  4 AU1 nucleic acid sequence
agcggccgcagcagtggacaaccaaaagcaccatcagtaccgaactccgcctcgcactctggcagcgcgcctaatacaagttcagctccggggtccgatacttatcgctacattagcgcttctagcggccagcctaaagctccgagtgtccccaattcagcgtcccattcggggtctgccccaaacacgtcgtccgcacccggttcagacacatacaggtatatttcgcgaagcgttggacaaccgaaagcaccctcggtgccaaactccgcatcacatagtggcagcgcccccaatacaagttcagcgccagggtccgacacctaccgctatatcgatatctctagcgggcagcctaaggctccctcagttcccaactctgcttcccactcggggtctgcgccaaatacctctagcgcccctggctctgatacatatcgctacattggcgccagtagcggccaacctaaagcaccttcagtgccaaattccgcatcgcattctgggtcggcccccaatacttcctcagcgccagggagcagcagtggcgcctagtagggccggcaaggccggatcc

SEQ ID NO: 32 - protein, 188 aa, Artificial Sequence
  Synthetic:  4 AU1 amino acid sequence
  misc_feature (184)..(185): Location of stop codon
SGRSSGQPKAPSVPNSASHSGSAPNTSSAPGSDTYRYISASSGQPKAPSVPNSASHSGSAPNTSSAPGSDTYRYISRSVGQPKAPSVPNSASHSGSAPNTSSAPGSDTYRYIDISSGQPKAPSVPNSASHSGSAPNTSSAPGSDTYRYIGASSGQPKAPSVPNSASHSGSAPNTSSAPGSSSGAGRQG